European Patent Specification EP 4 011 411 B1, published September 4, 2024. Title: Preparation Method for Silk Fibroin Nerve Graft Fused with NT3. Applicant: Nantong University. Application EP20935613.8. The sequence listing filed with the application follows.

SEQUENCE LISTING (4 sequences)

SEQ ID NO: 1 - protein, 253 aa, Artificial Sequence
  PEPTIDE, silk fibroin
MHHHHHHAPSVTINQYSDNEIPRDIDDGKASSVISRAWDYVDDTDKSIAILNVQEILKDMASQGDYASQASAVAQTAGIIAHLSAGIPGDACAAANVINSYTDGVRSGNFAGFRQSLGPFFGHVGQNLNLINQLVINPGQLRYSVGPALGCAGGGRIYDFEAAWDAILASSDSSFLNEEYCIVKRLYNSRNSQSNNIAAYITAHLLPPVAQVFHQSAGSITDLLRGVGNGNDATGLVANAQRYIAQAASQVHV

SEQ ID NO: 2 - protein, 372 aa, Artificial Sequence
  PEPTIDE, silk fibroin fused with NT3
MHHHHHHAPSVTINQYSDNEIPRDIDDGKASSVISRAWDYVDDTDKSIAILNVQEILKDMASQGDYASQASAVAQTAGIIAHLSAGIPGDACAAANVINSYTDGVRSGNFAGFRQSLGPFFGHVGQNLNLINQLVINPGQLRYSVGPALGCAGGGRIYDFEAAWDAILASSDSSFLNEEYCIVKRLYNSRNSQSNNIAAYITAHLLPPVAQVFHQSAGSITDLLRGVGNGNDATGLVANAQRYIAQAASQVHVYAEHKSHRGEYSVCDSESLWVTDKSSAIDIRGHQVTVLGEIKTGNSPVKQYFYETRCKEARPVKNGCRGIDDKHWNSQCKTSQTYVRALTSENNKLVGWRWIRIDTSCVCALSRKIGRT

SEQ ID NO: 3 - protein, 382 aa, Artificial Sequence
  PEPTIDE, silk fibroin fused with NT3
MHHHHHHAPSVTINQYSDNEIPRDIDDGKASSVISRAWDYVDDTDKSIAILNVQEILKDMASQGDYASQASAVAQTAGIIAHLSAGIPGDACAAANVINSYTDGVRSGNFAGFRQSLGPFFGHVGQNLNLINQLVINPGQLRYSVGPALGCAGGGRIYDFEAAWDAILASSDSSFLNEEYCIVKRLYNSRNSQSNNIAAYITAHLLPPVAQVFHQSAGSITDLLRGVGNGNDATGLVANAQRYIAQAASQVHVGGGGSGGGGSYAEHKSHRGEYSVCDSESLWVTDKSSAIDIRGHQVTVLGEIKTGNSPVKQYFYETRCKEARPVKNGCRGIDDKHWNSQCKTSQTYVRALTSENNKLVGWRWIRIDTSCVCALSRKIGRT

SEQ ID NO: 4 - protein, 501 aa, Artificial Sequence
  PEPTIDE, silk fibroin fused with NT3
MHHHHHHAPSVTINQYSDNEIPRDIDDGKASSVISRAWDYVDDTDKSIAILNVQEILKDMASQGDYASQASAVAQTAGIIAHLSAGIPGDACAAANVINSYTDGVRSGNFAGFRQSLGPFFGHVGQNLNLINQLVINPGQLRYSVGPALGCAGGGRIYDFEAAWDAILASSDSSFLNEEYCIVKRLYNSRNSQSNNIAAYITAHLLPPVAQVFHQSAGSITDLLRGVGNGNDATGLVANAQRYIAQAASQVHVYAEHKSHRGEYSVCDSESLWVTDKSSAIDIRGHQVTVLGEIKTGNSPVKQYFYETRCKEARPVKNGCRGIDDKHWNSQCKTSQTYVRALTSENNKLVGWRWIRIDTSCVCALSRKIGRTGGGGSGGGGSYAEHKSHRGEYSVCDSESLWVTDKSSAIDIRGHQVTVLGEIKTGNSPVKQYFYETRCKEARPVKNGCRGIDDKHWNSQCKTSQTYVRALTSENNKLVGWRWIRIDTSCVCALSRKIGRT